European Patent Specification EP 3 894 551 B1, published April 22, 2026. Title: Polypeptides Having Xylanase Activity And Polynucleotides Encoding Same. Applicant: Novoyzmes A/S Spodsberg, Nikolaj Osborn, David. The sequence listing filed with the application follows.

SEQUENCE LISTING (5 sequences)

SEQ ID NO: 1 - DNA, 1418 bp, Neosartorya massa
atggttcatctttcttcaatcgcagcagccttgactgctctgcccctgtatgttacctgctctcatgagaggagaaatggctctgacattgctacagcgtatatggagctggtctgaacacagcagctaaagccaaagggctaaagtacttcgggtccgctactgacaacccagagctcacggacactgcgtacgtcgctcaactgagcaacacagatgactttggtcaaatcactcccggaaactccatgaaggtttgtttacacctttgccctggaggatcccgtcaggagctaattgcgtactttggtggacagtgggatgccaccgagccttctcagaattctttctcgttcgcaaacggagacgctattgtcaatctggcgaacaagaatggccagatgatgcgatgccatactctggtctggcacagtcagcttcctaactggggtaagtggacgtctttttcattctcaattatctctaacggttgacagtctctagcggatcatggaccaatgcaacccttttggcggccatgaagaaccatatcactaacgtggttactcactacaaggggaagtgctatgcctgggatgttgtcaatgaaggttcgtttctccgtctatccttcaacagtactttcgaaactgacaagcctcaatatagccctgaacgaggacggtaccttccgtaactccatcttctaccagacaatcggcgaagcatacattcccattgcattcgcgactgccgccgcagcagaccccagcgtgaaactctactacaacgactacaacatcgaatactctggcgccaaagcgactgcagcgcagaacatcgtcaagatgatcaaggcctacggagcgaagattgacggcgtcggtctccagggccattttattctcggcagcactccaagccaatcggctctgacgagcgttttggagggctacactgctctcggcgtggaggtggcctataccgaacttgacatccgcatgcagctgccctcgaccgacgcaaagctggcccagcaggccacggagtaccagaacgtggctgcagcttgcgttggcaccactggctgtgtgggcgtcaccatctgggactggaccgacaagtactcctgggtccccagcgtgttctcaggctacggcgccgcattgccttgggatgagaactatgtgaagaagccagcatacaatggcattttggcggggcttggagcaagcggctccacgatgaccactaccttgactaccaccacgaagacctctactacgacaactgcgacgtctactggagtcgctcagaaatggggacagtgcggcggtatcggctggaccggcccaacaacctgcgtcagtgggactacctgccagaagttgaatgattggtactcgcagtgtctgtaa

SEQ ID NO: 2 - protein, 399 aa, Neosartorya massa
MVHLSSIAAALTALPLVYGAGLNTAAKAKGLKYFGSATDNPELTDTAYVAQLSNTDDFGQITPGNSMKWDATEPSQNSFSFANGDAIVNLANKNGQMMRCHTLVWHSQLPNWVSSGSWTNATLLAAMKNHITNVVTHYKGKCYAWDVVNEALNEDGTFRNSIFYQTIGEAYIPIAFATAAAADPSVKLYYNDYNIEYSGAKATAAQNIVKMIKAYGAKIDGVGLQGHFILGSTPSQSALTSVLEGYTALGVEVAYTELDIRMQLPSTDAKLAQQATEYQNVAAACVGTTGCVGVTIWDWTDKYSWVPSVFSGYGAALPWDENYVKKPAYNGILAGLGASGSTMTTTLTTTTKTSTTTTATSTGVAQKWGQCGGIGWTGPTTCVSGTTCQKLNDWYSQCL

SEQ ID NO: 3 - protein, 380 aa, Neosartorya massa
AGLNTAAKAKGLKYFGSATDNPELTDTAYVAQLSNTDDFGQITPGNSMKWDATEPSQNSFSFANGDAIVNLANKNGQMMRCHTLVWHSQLPNWVSSGSWTNATLLAAMKNHITNVVTHYKGKCYAWDVVNEALNEDGTFRNSIFYQTIGEAYIPIAFATAAAADPSVKLYYNDYNIEYSGAKATAAQNIVKMIKAYGAKIDGVGLQGHFILGSTPSQSALTSVLEGYTALGVEVAYTELDIRMQLPSTDAKLAQQATEYQNVAAACVGTTGCVGVTIWDWTDKYSWVPSVFSGYGAALPWDENYVKKPAYNGILAGLGASGSTMTTTLTTTTKTSTTTTATSTGVAQKWGQCGGIGWTGPTTCVSGTTCQKLNDWYSQCL

SEQ ID NO: 4 - DNA, 45 bp, Artificial Sequence
  Artificial DNA Primer
acacaactggggatccaccatggttcatctttcttcaatcgcagc

SEQ ID NO: 5 - DNA, 40 bp, Artificial Sequence
  Artificial DNA Primer
ccctctagatctcgagttacagacactgcgagtaccaatc